European Patent Specification EP 3 283 620 B1, published August 28, 2024. Title: MODIFIED GAMMA DELTA T CELLS AND USES THEREOF. Applicant: TC BIOPHARM LTD. The sequence listing filed with the application follows.

SEQUENCE LISTING (15 sequences)

SEQ ID NO: 1 - DNA, 1599 bp, Artificial Sequence
  Nucleic acid sequence of non-tuneable / classical CAR
atgcttctcctggtgacaagccttctgctctgtgagttaccacacccagcattcctcctgatcccagacatccagatgacacagactacatcctccctgtctgcctctctgggagacagagtcaccatcagttgcagggcaagtcaggacattagtaaatatttaaattggtatcagcagaaaccagatggaactgttaaactcctgatctaccatacatcaagattacactcaggagtcccatcaaggttcagtggcagtgggtctggaacagattattctctcaccattagcaacctggagcaagaagatattgccacttacttttgccaacagggtaatacgcttccgtacacgttcggaggggggactaagttggaaataacaggctccacctctggatccggcaagcccggatctggcgagggatccaccaagggcgaggtgaaactgcaggagtcaggacctggcctggtggcgccctcacagagcctgtccgtcacatgcactgtctcaggggtctcattacccgactatggtgtaagctggattcgccagcctccacgaaagggtctggagtggctgggagtaatatggggtagtgaaaccacatactataattcagctctcaaatccagactgaccatcatcaaggacaactccaagagccaagttttcttaaaaatgaacagtctgcaaactgatgacacagccatttactactgtgccaaacattattactacggtggtagctatgctatggactactggggtcaaggaacctcagtcaccgtctcctcagcggccgcaattgaagttatgtatcctcctccttacctagacaatgagaagagcaatggaaccattatccatgtgaaagggaaacacctttgtccaagtcccctatttcccggaccttctaagcccttttgggtgctggtggtggttgggggagtcctggcttgctatagcttgctagtaacagtggcctttattattttctgggtgaggagtaagaggagcaggctcctgcacagtgactacatgaacatgactccccgccgccccgggcccacccgcaagcattaccagccctatgccccaccacgcgacttcgcagcctatcgctccaaacggggcagaaagaaactcctgtatatattcaaacaaccatttatgagaccagtacaaactactcaagaggaagatggctgtagctgccgatttccagaagaagaagaaggaggatgtgaactgagagtgaagttcagcaggagcgcagacgcccccgcgtaccagcagggccagaaccagctctataacgagctcaatctaggacgaagagaggagtacgatgttttggacaagagacgtggccgggaccctgagatggggggaaagccgagaaggaagaaccctcaggaaggcctgtacaatgaactgcagaaagataagatggcggaggcctacagtgagattgggatgaaaggcgagcgccggaggggcaaggggcacgatggcctttaccagggtctcagtacagccaccaaggacacctacgacgcccttcacatgcaggccctgccccctcgctaatga

SEQ ID NO: 2 - protein, 22 aa, Artificial Sequence
  Secretion Signal
MLLLVTSLLLCELPHPAFLLIP

SEQ ID NO: 3 - protein, 248 aa, Artificial Sequence
  Anti-CD19 scFv
DIQMTQTTSSLSASLGDRVTISCRASQDISKYLNWYQQKPDGTVKLLIYHTSRLHSGVPSRFSGSGSGTDYSLTISNLEQEDIATYFCQQGNTLPYTFGGGTKLEITGSTSGSGKPGSGEGSTKGEVKLQESGPGLVAPSQSLSVTCTVSGVSLPDYGVSWIRQPPRKGLEWLGVIWGSETTYYNSALKSRLTIIKDNSKSQVFLKMNSLQTDDTAIYYCAKHYYYGGSYAMDYWGQGTSVTVSSAAA

SEQ ID NO: 4 - protein, 107 aa, Artificial Sequence
  CD28 hinge transmembrane domain co-stimulatory domain
IEVMYPPPYLDNEKSNGTIIHVKGKHLCPSPLFPGPSKPFWVLVVVGGVLACYSLLVTVAFIIFWVRSKRSRLLHSDYMNMTPRRPGPTRKHYQPYAPPRDFAAYRS

SEQ ID NO: 5 - protein, 42 aa, Artificial Sequence
  CD137 4-1BB co-stimulatory domain
KRGRKKLLYIFKQPFMRPVQTTQEEDGCSCRFPEEEEGGCEL

SEQ ID NO: 6 - protein, 112 aa, Artificial Sequence
  CD3 zeta activation domain
RVKFSRSADAPAYQQGQNQLYNELNLGRREEYDVLDKRRGRDPEMGGKPRRKNPQEGLYNELQKDKMAEAYSEIGMKGERRRGKGHDGLYQGLSTATKDTYDALHMQALPPR

SEQ ID NO: 7 - DNA, 1263 bp, Artificial Sequence
  Nucleic acid sequence of TCR-tuneable / co-stimulatory CAR
atgcttctcctggtgacaagccttctgctctgtgagttaccacacccagcattcctcctgatcccagacatccagatgacacagactacatcctccctgtctgcctctctgggagacagagtcaccatcagttgcagggcaagtcaggacattagtaaatatttaaattggtatcagcagaaaccagatggaactgttaaactcctgatctaccatacatcaagattacactcaggagtcccatcaaggttcagtggcagtgggtctggaacagattattctctcaccattagcaacctggagcaagaagatattgccacttacttttgccaacagggtaatacgcttccgtacacgttcggaggggggactaagttggaaataacaggctccacctctggatccggcaagcccggatctggcgagggatccaccaagggcgaggtgaaactgcaggagtcaggacctggcctggtggcgccctcacagagcctgtccgtcacatgcactgtctcaggggtctcattacccgactatggtgtaagctggattcgccagcctccacgaaagggtctggagtggctgggagtaatatggggtagtgaaaccacatactataattcagctctcaaatccagactgaccatcatcaaggacaactccaagagccaagttttcttaaaaatgaacagtctgcaaactgatgacacagccatttactactgtgccaaacattattactacggtggtagctatgctatggactactggggtcaaggaacctcagtcaccgtctcctcagcggccgcaattgaagttatgtatcctcctccttacctagacaatgagaagagcaatggaaccattatccatgtgaaagggaaacacctttgtccaagtcccctatttcccggaccttctaagcccttttgggtgctggtggtggttgggggagtcctggcttgctatagcttgctagtaacagtggcctttattattttctgggtgaggagtaagaggagcaggctcctgcacagtgactacatgaacatgactccccgccgccccgggcccacccgcaagcattaccagccctatgccccaccacgcgacttcgcagcctatcgctccaaacggggcagaaagaaactcctgtatatattcaaacaaccatttatgagaccagtacaaactactcaagaggaagatggctgtagctgccgatttccagaagaagaagaaggaggatgtgaactgtaatga

SEQ ID NO: 8 - protein, 22 aa, Artificial Sequence
  Secretion signal
MLLLVTSLLLCELPHPAFLLIP

SEQ ID NO: 9 - protein, 248 aa, Artificial Sequence; identical to SEQ ID NO: 3
  Anti-CD19 scFv

SEQ ID NO: 10 - protein, 107 aa, Artificial Sequence; identical to SEQ ID NO: 4
  CD28 hinge transmembrane domain co-stimulatory domain

SEQ ID NO: 11 - protein, 42 aa, Artificial Sequence; identical to SEQ ID NO: 5
  CD137 4-1BB co-stimulatory domain

SEQ ID NO: 12 - DNA, 21 bp, Artificial Sequence
  Universal primer - forward
gctcctgcacagtgactacat

SEQ ID NO: 13 - DNA, 20 bp, Artificial Sequence
  Universal primer - reverse
ggagtttctttctgccccgt

SEQ ID NO: 14 - DNA, 21 bp, Artificial Sequence
  Discriminatory primer - forward
ctgtagctgccgatttccaga

SEQ ID NO: 15 - DNA, 22 bp, Artificial Sequence
  Discriminatory primer - reverse
catcgtactcctctcttcgtcc